European Patent Specification EP 3 313 443 B9, published October 4, 2023. Title: COMBINING ANTI-HLA-DR OR ANTI-TROP-2 ANTIBODIES WITH MICROTUBULE INHIBITORS, PARP INHIBITORS, BRUTON KINASE INHIBITORS OR PHOSPHOINOSITIDE 3-KINASE INHIBITORS SIGNIFICANTLY IMPROVES THERAPEUTIC OUTCOME IN CANCER. Applicant: IMMUNOMEDICS, INC. The sequence listing filed with the application follows.

SEQUENCE LISTING (161 sequences)

SEQ ID NO: 1 - protein, 44 aa, Artificial Sequence
  Description of Artificial Sequence: Synthetic polypeptide
SHIQIPPGLTELLQGYTVEVLRQQPPDLVEFAVEYFTRLREARA

SEQ ID NO: 2 - protein, 45 aa, Artificial Sequence
  Description of Artificial Sequence: Synthetic polypeptide
CGHIQIPPGLTELLQGYTVEVLRQQPPDLVEFAVEYFTRLREARA

SEQ ID NO: 3 - protein, 17 aa, Artificial Sequence
  Description of Artificial Sequence: Synthetic peptide
QIEYLAKQIVDNAIQQA

SEQ ID NO: 4 - protein, 21 aa, Artificial Sequence
  Description of Artificial Sequence: Synthetic peptide
CGQIEYLAKQIVDNAIQQAGC

SEQ ID NO: 5 - protein, 50 aa, Artificial Sequence
  Description of Artificial Sequence: Synthetic polypeptide
SLRECELYVQKHNIQALLKDSIVQLCTARPERPMAFLREYFERLEKEEAK

SEQ ID NO: 6 - protein, 55 aa, Artificial Sequence
  Description of Artificial Sequence: Synthetic polypeptide
MSCGGSLRECELYVQKHNIQALLKDSIVQLCTARPERPMAFLREYFERLEKEEAK

SEQ ID NO: 7 - protein, 23 aa, Artificial Sequence
  Description of Artificial Sequence: Synthetic peptide
CGFEELAWKIAKMIWSDVFQQGC

SEQ ID NO: 8 - protein, 51 aa, Artificial Sequence
  Description of Artificial Sequence: Synthetic polypeptide
SLRECELYVQKHNIQALLKDVSIVQLCTARPERPMAFLREYFEKLEKEEAK

SEQ ID NO: 9 - protein, 54 aa, Artificial Sequence
  Description of Artificial Sequence: Synthetic polypeptide
SLKGCELYVQLHGIQQVLKDCIVHLCISKPERPMKFLREHFEKLEKEENRQILA

SEQ ID NO: 10 - protein, 44 aa, Artificial Sequence
  Description of Artificial Sequence: Synthetic polypeptide
SHIQIPPGLTELLQGYTVEVGQQPPDLVDFAVEYFTRLREARRQ

SEQ ID NO: 11 - protein, 44 aa, Artificial Sequence
  Description of Artificial Sequence: Synthetic polypeptide
SIEIPAGLTELLQGFTVEVLRHQPADLLEFALQHFTRLQQENER

SEQ ID NO: 12 - protein, 44 aa, Artificial Sequence
  Description of Artificial Sequence: Synthetic polypeptide
THIQIPPGLTELLQGYTVEVLRQQPPDLVEFAVEYFTRLREARA

SEQ ID NO: 13 - protein, 44 aa, Artificial Sequence
  Description of Artificial Sequence: Synthetic polypeptide
SKIQIPPGLTELLQGYTVEVLRQQPPDLVEFAVEYFTRLREARA

SEQ ID NO: 14 - protein, 44 aa, Artificial Sequence
  Description of Artificial Sequence: Synthetic polypeptide
SRIQIPPGLTELLQGYTVEVLRQQPPDLVEFAVEYFTRLREARA

SEQ ID NO: 15 - protein, 44 aa, Artificial Sequence
  Description of Artificial Sequence: Synthetic polypeptide
SHINIPPGLTELLQGYTVEVLRQQPPDLVEFAVEYFTRLREARA

SEQ ID NO: 16 - protein, 44 aa, Artificial Sequence
  Description of Artificial Sequence: Synthetic polypeptide
SHIQIPPALTELLQGYTVEVLRQQPPDLVEFAVEYFTRLREARA

SEQ ID NO: 17 - protein, 44 aa, Artificial Sequence
  Description of Artificial Sequence: Synthetic polypeptide
SHIQIPPGLSELLQGYTVEVLRQQPPDLVEFAVEYFTRLREARA

SEQ ID NO: 18 - protein, 44 aa, Artificial Sequence
  Description of Artificial Sequence: Synthetic polypeptide
SHIQIPPGLTDLLQGYTVEVLRQQPPDLVEFAVEYFTRLREARA

SEQ ID NO: 19 - protein, 44 aa, Artificial Sequence
  Description of Artificial Sequence: Synthetic polypeptide
SHIQIPPGLTELLNGYTVEVLRQQPPDLVEFAVEYFTRLREARA

SEQ ID NO: 20 - protein, 44 aa, Artificial Sequence
  Description of Artificial Sequence: Synthetic polypeptide
SHIQIPPGLTELLQAYTVEVLRQQPPDLVEFAVEYFTRLREARA

SEQ ID NO: 21 - protein, 44 aa, Artificial Sequence
  Description of Artificial Sequence: Synthetic polypeptide
SHIQIPPGLTELLQGYSVEVLRQQPPDLVEFAVEYFTRLREARA

SEQ ID NO: 22 - protein, 44 aa, Artificial Sequence
  Description of Artificial Sequence: Synthetic polypeptide
SHIQIPPGLTELLQGYTVDVLRQQPPDLVEFAVEYFTRLREARA

SEQ ID NO: 23 - protein, 44 aa, Artificial Sequence
  Description of Artificial Sequence: Synthetic polypeptide
SHIQIPPGLTELLQGYTVEVLKQQPPDLVEFAVEYFTRLREARA

SEQ ID NO: 24 - protein, 44 aa, Artificial Sequence
  Description of Artificial Sequence: Synthetic polypeptide
SHIQIPPGLTELLQGYTVEVLRNQPPDLVEFAVEYFTRLREARA

SEQ ID NO: 25 - protein, 44 aa, Artificial Sequence
  Description of Artificial Sequence: Synthetic polypeptide
SHIQIPPGLTELLQGYTVEVLRQNPPDLVEFAVEYFTRLREARA

SEQ ID NO: 26 - protein, 44 aa, Artificial Sequence
  Description of Artificial Sequence: Synthetic polypeptide
SHIQIPPGLTELLQGYTVEVLRQQPPELVEFAVEYFTRLREARA

SEQ ID NO: 27 - protein, 44 aa, Artificial Sequence
  Description of Artificial Sequence: Synthetic polypeptide
SHIQIPPGLTELLQGYTVEVLRQQPPDLVDFAVEYFTRLREARA

SEQ ID NO: 28 - protein, 44 aa, Artificial Sequence
  Description of Artificial Sequence: Synthetic polypeptide
SHIQIPPGLTELLQGYTVEVLRQQPPDLVEFLVEYFTRLREARA

SEQ ID NO: 29 - protein, 44 aa, Artificial Sequence
  Description of Artificial Sequence: Synthetic polypeptide
SHIQIPPGLTELLQGYTVEVLRQQPPDLVEFIVEYFTRLREARA

SEQ ID NO: 30 - protein, 44 aa, Artificial Sequence
  Description of Artificial Sequence: Synthetic polypeptide
SHIQIPPGLTELLQGYTVEVLRQQPPDLVEFVVEYFTRLREARA

SEQ ID NO: 31 - protein, 44 aa, Artificial Sequence
  Description of Artificial Sequence: Synthetic polypeptide
SHIQIPPGLTELLQGYTVEVLRQQPPDLVEFAVDYFTRLREARA

SEQ ID NO: 32 - protein, 17 aa, Artificial Sequence
  Description of Artificial Sequence: Synthetic peptide
NIEYLAKQIVDNAIQQA

SEQ ID NO: 33 - protein, 17 aa, Artificial Sequence
  Description of Artificial Sequence: Synthetic peptide
QLEYLAKQIVDNAIQQA

SEQ ID NO: 34 - protein, 17 aa, Artificial Sequence
  Description of Artificial Sequence: Synthetic peptide
QVEYLAKQIVDNAIQQA

SEQ ID NO: 35 - protein, 17 aa, Artificial Sequence
  Description of Artificial Sequence: Synthetic peptide
QIDYLAKQIVDNAIQQA

SEQ ID NO: 36 - protein, 17 aa, Artificial Sequence
  Description of Artificial Sequence: Synthetic peptide
QIEFLAKQIVDNAIQQA

SEQ ID NO: 37 - protein, 17 aa, Artificial Sequence
  Description of Artificial Sequence: Synthetic peptide
QIETLAKQIVDNAIQQA

SEQ ID NO: 38 - protein, 17 aa, Artificial Sequence
  Description of Artificial Sequence: Synthetic peptide
QIESLAKQIVDNAIQQA

SEQ ID NO: 39 - protein, 17 aa, Artificial Sequence
  Description of Artificial Sequence: Synthetic peptide
QIEYIAKQIVDNAIQQA

SEQ ID NO: 40 - protein, 17 aa, Artificial Sequence
  Description of Artificial Sequence: Synthetic peptide
QIEYVAKQIVDNAIQQA

SEQ ID NO: 41 - protein, 17 aa, Artificial Sequence
  Description of Artificial Sequence: Synthetic peptide
QIEYLARQIVDNAIQQA

SEQ ID NO: 42 - protein, 17 aa, Artificial Sequence
  Description of Artificial Sequence: Synthetic peptide
QIEYLAKNIVDNAIQQA

SEQ ID NO: 43 - protein, 17 aa, Artificial Sequence
  Description of Artificial Sequence: Synthetic peptide
QIEYLAKQIVENAIQQA

SEQ ID NO: 44 - protein, 17 aa, Artificial Sequence
  Description of Artificial Sequence: Synthetic peptide
QIEYLAKQIVDQAIQQA

SEQ ID NO: 45 - protein, 17 aa, Artificial Sequence
  Description of Artificial Sequence: Synthetic peptide
QIEYLAKQIVDNAINQA

SEQ ID NO: 46 - protein, 17 aa, Artificial Sequence
  Description of Artificial Sequence: Synthetic peptide
QIEYLAKQIVDNAIQNA

SEQ ID NO: 47 - protein, 17 aa, Artificial Sequence
  Description of Artificial Sequence: Synthetic peptide
QIEYLAKQIVDNAIQQL

SEQ ID NO: 48 - protein, 17 aa, Artificial Sequence
  Description of Artificial Sequence: Synthetic peptide
QIEYLAKQIVDNAIQQI

SEQ ID NO: 49 - protein, 17 aa, Artificial Sequence
  Description of Artificial Sequence: Synthetic peptide
QIEYLAKQIVDNAIQQV

SEQ ID NO: 50 - protein, 17 aa, Artificial Sequence
  Description of Artificial Sequence: Synthetic peptide
QIEYVAKQIVDYAIHQA

SEQ ID NO: 51 - protein, 17 aa, Artificial Sequence
  Description of Artificial Sequence: Synthetic peptide
QIEYKAKQIVDHAIHQA

SEQ ID NO: 52 - protein, 17 aa, Artificial Sequence
  Description of Artificial Sequence: Synthetic peptide
QIEYHAKQIVDHAIHQA

SEQ ID NO: 53 - protein, 17 aa, Artificial Sequence
  Description of Artificial Sequence: Synthetic peptide
QIEYVAKQIVDHAIHQA

SEQ ID NO: 54 - protein, 18 aa, Artificial Sequence
  Description of Artificial Sequence: Synthetic peptide
PLEYQAGLLVQNAIQQAI

SEQ ID NO: 55 - protein, 18 aa, Artificial Sequence
  Description of Artificial Sequence: Synthetic peptide
LLIETASSLVKNAIQLSI

SEQ ID NO: 56 - protein, 18 aa, Artificial Sequence
  Description of Artificial Sequence: Synthetic peptide
LIEEAASRIVDAVIEQVK

SEQ ID NO: 57 - protein, 18 aa, Artificial Sequence
  Description of Artificial Sequence: Synthetic peptide
ALYQFADRFSELVISEAL

SEQ ID NO: 58 - protein, 17 aa, Artificial Sequence
  Description of Artificial Sequence: Synthetic peptide
LEQVANQLADQIIKEAT

SEQ ID NO: 59 - protein, 17 aa, Artificial Sequence
  Description of Artificial Sequence: Synthetic peptide
FEELAWKIAKMIWSDVF

SEQ ID NO: 60 - protein, 18 aa, Artificial Sequence
  Description of Artificial Sequence: Synthetic peptide
ELVRLSKRLVENAVLKAV

SEQ ID NO: 61 - protein, 18 aa, Artificial Sequence
  Description of Artificial Sequence: Synthetic peptide
TAEEVSARIVQVVTAEAV

SEQ ID NO: 62 - protein, 18 aa, Artificial Sequence
  Description of Artificial Sequence: Synthetic peptide
QIKQAAFQLISQVILEAT

SEQ ID NO: 63 - protein, 16 aa, Artificial Sequence
  Description of Artificial Sequence: Synthetic peptide
LAWKIAKMIVSDVMQQ

SEQ ID NO: 64 - protein, 24 aa, Artificial Sequence
  Description of Artificial Sequence: Synthetic peptide
DLIEEAASRIVDAVIEQVKAAGAY

SEQ ID NO: 65 - protein, 18 aa, Artificial Sequence
  Description of Artificial Sequence: Synthetic peptide
LEQYANQLADQIIKEATE

SEQ ID NO: 66 - protein, 20 aa, Artificial Sequence
  Description of Artificial Sequence: Synthetic peptide
FEELAWKIAKMIWSDVFQQC

SEQ ID NO: 67 - protein, 17 aa, Artificial Sequence
  Description of Artificial Sequence: Synthetic peptide
QIEYLAKQIPDNAIQQA

SEQ ID NO: 68 - protein, 25 aa, Artificial Sequence
  Description of Artificial Sequence: Synthetic peptide
KGADLIEEAASRIVDAVIEQVKAAG

SEQ ID NO: 69 - protein, 25 aa, Artificial Sequence
  Description of Artificial Sequence: Synthetic peptide
KGADLIEEAASRIPDAPIEQVKAAG

SEQ ID NO: 70 - protein, 25 aa, Artificial Sequence
  Description of Artificial Sequence: Synthetic peptide
PEDAELVRLSKRLVENAVLKAVQQY

SEQ ID NO: 71 - protein, 25 aa, Artificial Sequence
  Description of Artificial Sequence: Synthetic peptide
PEDAELVRTSKRLVENAVLKAVQQY

SEQ ID NO: 72 - protein, 25 aa, Artificial Sequence
  Description of Artificial Sequence: Synthetic peptide
PEDAELVRLSKRDVENAVLKAVQQY

SEQ ID NO: 73 - protein, 25 aa, Artificial Sequence
  Description of Artificial Sequence: Synthetic peptide
PEDAELVRLSKRLPENAVLKAVQQY

SEQ ID NO: 74 - protein, 25 aa, Artificial Sequence
  Description of Artificial Sequence: Synthetic peptide
PEDAELVRLSKRLPENAPLKAVQQY

SEQ ID NO: 75 - protein, 25 aa, Artificial Sequence
  Description of Artificial Sequence: Synthetic peptide
PEDAELVRLSKRLVENAVEKAVQQY

SEQ ID NO: 76 - protein, 25 aa, Artificial Sequence
  Description of Artificial Sequence: Synthetic peptide
EEGLDRNEEIKRAAFQIISQVISEA

SEQ ID NO: 77 - protein, 25 aa, Artificial Sequence
  Description of Artificial Sequence: Synthetic peptide
LVDDPLEYQAGLLVQNAIQQAIAEQ

SEQ ID NO: 78 - protein, 25 aa, Artificial Sequence
  Description of Artificial Sequence: Synthetic peptide
QYETLLIETASSLVKNAIQLSIEQL

SEQ ID NO: 79 - protein, 25 aa, Artificial Sequence
  Description of Artificial Sequence: Synthetic peptide
LEKQYQEQLEEEVAKVIVSMSIAFA

SEQ ID NO: 80 - protein, 25 aa, Artificial Sequence
  Description of Artificial Sequence: Synthetic peptide
NTDEAQEELAWKIAKMIVSDIMQQA

SEQ ID NO: 81 - protein, 25 aa, Artificial Sequence
  Description of Artificial Sequence: Synthetic peptide
VNLDKKAVLAEKIVAEAIEKAEREL

SEQ ID NO: 82 - protein, 25 aa, Artificial Sequence
  Description of Artificial Sequence: Synthetic peptide
NGILELETKSSKLVQNIIQTAVDQF

SEQ ID NO: 83 - protein, 25 aa, Artificial Sequence
  Description of Artificial Sequence: Synthetic peptide
TQDKNYEDELTQVALALVEDVINYA

SEQ ID NO: 84 - protein, 25 aa, Artificial Sequence
  Description of Artificial Sequence: Synthetic peptide
ETSAKDNINIEEAARFLVEKILVNH

SEQ ID NO: 85 - protein, 330 aa, Artificial Sequence
  Description of Artificial Sequence: Synthetic polypeptide
ASTKGPSVFPLAPSSKSTSGGTAALGCLVKDYFPEPVTVSWNSGALTSGVHTFPAVLQSSGLYSLSSVVTVPSSSLGTQTYICNVNHKPSNTKVDKKAEPKSCDKTHTCPPCPAPELLGGPSVFLFPPKPKDTLMISRTPEVTCVVVDVSHEDPEVKFNWYVDGVEVHNAKTKPREEQYNSTYRVVSVLTVLHQDWLNGKEYKCKVSNKALPAPIEKTISKAKGQPREPQVYTLPPSRDELTKNQVSLTCLVKGFYPSDIAVEWESNGQPENNYKTTPPVLDSDGSFFLYSKLTVDKSRWQQGNVFSCSVMHEALHNHYTQKSLSLSPGK

SEQ ID NO: 86 - protein, 330 aa, Artificial Sequence
  Description of Artificial Sequence: Synthetic polypeptide
ASTKGPSVFPLAPSSKSTSGGTAALGCLVKDYFPEPVTVSWNSGALTSGVHTFPAVLQSSGLYSLSSVVTVPSSSLGTQTYICNVNHKPSNTKVDKRVEPKSCDKTHTCPPCPAPELLGGPSVFLFPPKPKDTLMISRTPEVTCVVVDVSHEDPEVKFNWYVDGVEVHNAKTKPREEQYNSTYRVVSVLTVLHQDWLNGKEYKCKVSNKALPAPIEKTISKAKGQPREPQVYTLPPSREEMTKNQVSLTCLVKGFYPSDIAVEWESNGQPENNYKTTPPVLDSDGSFFLYSKLTVDKSRWQQGNVFSCSVMHEALHNHYTQKSLSLSPGK

SEQ ID NO: 87 - protein, 44 aa, Artificial Sequence
  Description of Artificial Sequence: Synthetic consensus polypeptide
  MOD_RES (1)..(1): Ser or Thr
  MOD_RES (2)..(2): His, Lys or Arg
  MOD_RES (4)..(4): Gln or Asn
  MOD_RES (8)..(8): Gly or Ala
  MOD_RES (10)..(10): Thr or Ser
  MOD_RES (11)..(11): Glu or Asp
  MOD_RES (14)..(14): Gln or Asn
  MOD_RES (15)..(15): Gly or Ala
  MOD_RES (17)..(17): Thr or Ser
  MOD_RES (19)..(19): Glu or Asp
  MOD_RES (22)..(22): Arg or Lys
  MOD_RES (23)..(24): Asn or Gln
  MOD_RES (27)..(27): Asp or Glu
  MOD_RES (30)..(30): Glu or Asp
  MOD_RES (32)..(32): Ala, Leu, Ile or Val
  MOD_RES (34)..(34): Glu or Asp
  MOD_RES (37)..(37): Thr or Ser
  MOD_RES (38)..(38): Arg or Lys
  MOD_RES (40)..(40): Arg or Lys
  MOD_RES (41)..(41): Glu or Asp
  MOD_RES (42)..(42): Ala, Leu, Ile or Val
  MOD_RES (43)..(43): Arg or Lys
  MOD_RES (44)..(44): Ala, Leu, Ile or Val
XXIXIPPXLXXLLXXYXVXVLXXXPPXLVXFXVXYFXXLXXXXX

SEQ ID NO: 88 - protein, 17 aa, Artificial Sequence
  Description of Artificial Sequence: Synthetic consensus peptide
  MOD_RES (1)..(1): Gln or Asn
  MOD_RES (2)..(2): Ile, Leu or Val
  MOD_RES (3)..(3): Glu or Asp
  MOD_RES (4)..(4): Tyr, Phe, Thr or Ser
  MOD_RES (5)..(5): Leu, Ile or Val
  MOD_RES (7)..(7): Lys or Arg
  MOD_RES (8)..(8): Gln or Asn
  MOD_RES (11)..(11): Asp or Glu
  MOD_RES (12)..(12): Asn or Gln
  MOD_RES (15)..(16): Gln or Asn
  MOD_RES (17)..(17): Ala, Leu, Ile or Val
XXXXXAXXIVXXAIXXX

SEQ ID NO: 89 - protein, 44 aa, Artificial Sequence
  Description of Artificial Sequence: Synthetic consensus polypeptide
  MOD_RES (1)..(1): Ser or Thr
  MOD_RES (4)..(4): Gln or Asn
  MOD_RES (10)..(10): Thr or Ser
  MOD_RES (18)..(18): Val, Ile, Leu or Ala
  MOD_RES (23)..(23): Gln or Asn
  MOD_RES (33)..(33): Val, Ile, Leu or Ala
  MOD_RES (34)..(34): Glu or Asp
  MOD_RES (37)..(37): Thr or Ser
  MOD_RES (38)..(38): Arg or Lys
  MOD_RES (40)..(40): Arg or Lys
  MOD_RES (42)..(42): Ala, Leu, Ile or Val
  MOD_RES (44)..(44): Ala, Leu, Ile or Val
XHIXIPPGLXELLQGYTXEVLRXQPPDLVEFAXXYFXXLXEXRX

SEQ ID NO: 90 - protein, 11 aa, Artificial Sequence
  Description of Artificial Sequence: Synthetic peptide
KASQDVSIAVA

SEQ ID NO: 91 - protein, 7 aa, Artificial Sequence
  Description of Artificial Sequence: Synthetic peptide
SASYRYT

SEQ ID NO: 92 - protein, 9 aa, Artificial Sequence
  Description of Artificial Sequence: Synthetic peptide
QQHYITPLT

SEQ ID NO: 93 - protein, 5 aa, Artificial Sequence
  Description of Artificial Sequence: Synthetic peptide
NYGMN

SEQ ID NO: 94 - protein, 17 aa, Artificial Sequence
  Description of Artificial Sequence: Synthetic peptide
WINTYTGEPTYTDDFKG

SEQ ID NO: 95 - protein, 12 aa, Artificial Sequence
  Description of Artificial Sequence: Synthetic peptide
GGFGSSYWYFDV

SEQ ID NO: 96 - protein, 11 aa, Artificial Sequence
  Description of Artificial Sequence: Synthetic peptide
KASQDVGTSVA

SEQ ID NO: 97 - protein, 7 aa, Artificial Sequence
  Description of Artificial Sequence: Synthetic peptide
WTSTRHT

SEQ ID NO: 98 - protein, 8 aa, Artificial Sequence
  Description of Artificial Sequence: Synthetic peptide
QQYSLYRS

SEQ ID NO: 99 - protein, 5 aa, Artificial Sequence
  Description of Artificial Sequence: Synthetic peptide
TYWMS

SEQ ID NO: 100 - protein, 17 aa, Artificial Sequence
  Description of Artificial Sequence: Synthetic peptide
EIHPDSSTINYAPSLKD

SEQ ID NO: 101 - protein, 10 aa, Artificial Sequence
  Description of Artificial Sequence: Synthetic peptide
LYFGFPWFAY

SEQ ID NO: 102 - protein, 16 aa, Artificial Sequence
  Description of Artificial Sequence: Synthetic peptide
RSSQSIVHSNGNTYLE

SEQ ID NO: 103 - protein, 7 aa, Artificial Sequence
  Description of Artificial Sequence: Synthetic peptide
KVSNRFS

SEQ ID NO: 104 - protein, 9 aa, Artificial Sequence
  Description of Artificial Sequence: Synthetic peptide
FQGSHVPPT

SEQ ID NO: 105 - protein, 5 aa, Artificial Sequence
  Description of Artificial Sequence: Synthetic peptide
NYGMN

SEQ ID NO: 106 - protein, 17 aa, Artificial Sequence
  Description of Artificial Sequence: Synthetic peptide
WINTYTGEPTYADDFKG

SEQ ID NO: 107 - protein, 12 aa, Artificial Sequence
  Description of Artificial Sequence: Synthetic peptide
KGWMDFNSSLDY

SEQ ID NO: 108 - protein, 10 aa, Artificial Sequence
  Description of Artificial Sequence: Synthetic peptide
SASSRVSYIH

SEQ ID NO: 109 - protein, 7 aa, Artificial Sequence
  Description of Artificial Sequence: Synthetic peptide
GTSTLAS

SEQ ID NO: 110 - protein, 9 aa, Artificial Sequence
  Description of Artificial Sequence: Synthetic peptide
QQWSYNPPT

SEQ ID NO: 111 - protein, 5 aa, Artificial Sequence
  Description of Artificial Sequence: Synthetic peptide
DYYMS

SEQ ID NO: 112 - protein, 19 aa, Artificial Sequence
  Description of Artificial Sequence: Synthetic peptide
FIANKANGHTTDYSPSVKG

SEQ ID NO: 113 - protein, 10 aa, Artificial Sequence
  Description of Artificial Sequence: Synthetic peptide
DMGIRWNFDV

SEQ ID NO: 114 - protein, 16 aa, Artificial Sequence
  Description of Artificial Sequence: Synthetic peptide
RSSQSLVHRNGNTYLH

SEQ ID NO: 115 - protein, 7 aa, Artificial Sequence
  Description of Artificial Sequence: Synthetic peptide
TVSNRFS

SEQ ID NO: 116 - protein, 9 aa, Artificial Sequence
  Description of Artificial Sequence: Synthetic peptide
SQSSHVPPT

SEQ ID NO: 117 - protein, 5 aa, Artificial Sequence
  Description of Artificial Sequence: Synthetic peptide
NYGVN

SEQ ID NO: 118 - protein, 17 aa, Artificial Sequence
  Description of Artificial Sequence: Synthetic peptide
WINPNTGEPTFDDDFKG

SEQ ID NO: 119 - protein, 11 aa, Artificial Sequence
  Description of Artificial Sequence: Synthetic peptide
SRGKNEAWFAY

SEQ ID NO: 120 - protein, 16 aa, Artificial Sequence
  Description of Artificial Sequence: Synthetic peptide
KSSQSVLYSANHKYLA

SEQ ID NO: 121 - protein, 7 aa, Artificial Sequence
  Description of Artificial Sequence: Synthetic peptide
WASTRES

SEQ ID NO: 122 - protein, 9 aa, Artificial Sequence
  Description of Artificial Sequence: Synthetic peptide
HQYLSSWTF

SEQ ID NO: 123 - protein, 5 aa, Artificial Sequence
  Description of Artificial Sequence: Synthetic peptide
SYWLH

SEQ ID NO: 124 - protein, 17 aa, Artificial Sequence
  Description of Artificial Sequence: Synthetic peptide
YINPRNDYTEYNQNFKD

SEQ ID NO: 125 - protein, 7 aa, Artificial Sequence
  Description of Artificial Sequence: Synthetic peptide
RDITTFY

SEQ ID NO: 126 - protein, 16 aa, Artificial Sequence
  Description of Artificial Sequence: Synthetic peptide
RSSQSIVHSNGNTYLE

SEQ ID NO: 127 - protein, 7 aa, Artificial Sequence
  Description of Artificial Sequence: Synthetic peptide
KVSNRFS

SEQ ID NO: 128 - protein, 9 aa, Artificial Sequence
  Description of Artificial Sequence: Synthetic peptide
FQGSRVPYT

SEQ ID NO: 129 - protein, 5 aa, Artificial Sequence
  Description of Artificial Sequence: Synthetic peptide
EYVIT

SEQ ID NO: 130 - protein, 16 aa, Artificial Sequence
  Description of Artificial Sequence: Synthetic peptide
EIYPGSGSTSYNEKFK

SEQ ID NO: 131 - protein, 3 aa, Artificial Sequence
  Description of Artificial Sequence: Synthetic peptide
EDL

SEQ ID NO: 132 - protein, 12 aa, Artificial Sequence
  Description of Artificial Sequence: Synthetic peptide
SASSSVSSSYLY

SEQ ID NO: 133 - protein, 7 aa, Artificial Sequence
  Description of Artificial Sequence: Synthetic peptide
STSNLAS

SEQ ID NO: 134 - protein, 9 aa, Artificial Sequence
  Description of Artificial Sequence: Synthetic peptide
HQWNRYPYT

SEQ ID NO: 135 - protein, 5 aa, Artificial Sequence
  Description of Artificial Sequence: Synthetic peptide
SYVLH

SEQ ID NO: 136 - protein, 17 aa, Artificial Sequence
  Description of Artificial Sequence: Synthetic peptide
YINPYNDGTQYNEKFKG

SEQ ID NO: 137 - protein, 10 aa, Artificial Sequence
  Description of Artificial Sequence: Synthetic peptide
GFGGSYGFAY

SEQ ID NO: 138 - protein, 5 aa, Artificial Sequence
  Description of Artificial Sequence: Synthetic peptide
SYVIH

SEQ ID NO: 139 - protein, 17 aa, Artificial Sequence
  Description of Artificial Sequence: Synthetic peptide
YIHPYNGGTKYNEKFKG

SEQ ID NO: 140 - protein, 9 aa, Artificial Sequence
  Description of Artificial Sequence: Synthetic peptide
SGGGDPFAY

SEQ ID NO: 141 - protein, 11 aa, Artificial Sequence
  Description of Artificial Sequence: Synthetic peptide
KASQDINKYIG

SEQ ID NO: 142 - protein, 7 aa, Artificial Sequence
  Description of Artificial Sequence: Synthetic peptide
YTSALLP

SEQ ID NO: 143 - protein, 8 aa, Artificial Sequence
  Description of Artificial Sequence: Synthetic peptide
LQYDDLWT

SEQ ID NO: 144 - protein, 5 aa, Artificial Sequence
  Description of Artificial Sequence: Synthetic peptide
NYGMN

SEQ ID NO: 145 - protein, 17 aa, Artificial Sequence
  Description of Artificial Sequence: Synthetic peptide
WINTYTREPTYADDFKG

SEQ ID NO: 146 - protein, 12 aa, Artificial Sequence
  Description of Artificial Sequence: Synthetic peptide
DITAVVPTGFDY

SEQ ID NO: 147 - protein, 11 aa, Artificial Sequence
  Description of Artificial Sequence: Synthetic peptide
RASENIYSNLA

SEQ ID NO: 148 - protein, 7 aa, Artificial Sequence
  Description of Artificial Sequence: Synthetic peptide
AASNLAD

SEQ ID NO: 149 - protein, 9 aa, Artificial Sequence
  Description of Artificial Sequence: Synthetic peptide
QHFWTTPWA

SEQ ID NO: 150 - protein, 10 aa, Artificial Sequence
  Description of Artificial Sequence: Synthetic peptide
RASSSVSYIH

SEQ ID NO: 151 - protein, 7 aa, Artificial Sequence
  Description of Artificial Sequence: Synthetic peptide
ATSNLAS

SEQ ID NO: 152 - protein, 9 aa, Artificial Sequence
  Description of Artificial Sequence: Synthetic peptide
QQWTSNPPT

SEQ ID NO: 153 - protein, 5 aa, Artificial Sequence
  Description of Artificial Sequence: Synthetic peptide
SYNMH

SEQ ID NO: 154 - protein, 17 aa, Artificial Sequence
  Description of Artificial Sequence: Synthetic peptide
AIYPGNGDTSYNQKFKG

SEQ ID NO: 155 - protein, 12 aa, Artificial Sequence
  Description of Artificial Sequence: Synthetic peptide
STYYGGDWYFDV

SEQ ID NO: 156 - protein, 15 aa, Artificial Sequence
  Description of Artificial Sequence: Synthetic peptide
KASQSVDYDGDSYLN

SEQ ID NO: 157 - protein, 7 aa, Artificial Sequence
  Description of Artificial Sequence: Synthetic peptide
DASNLVS

SEQ ID NO: 158 - protein, 9 aa, Artificial Sequence
  Description of Artificial Sequence: Synthetic peptide
QQSTEDPWT

SEQ ID NO: 159 - protein, 5 aa, Artificial Sequence
  Description of Artificial Sequence: Synthetic peptide
SYWMN

SEQ ID NO: 160 - protein, 17 aa, Artificial Sequence
  Description of Artificial Sequence: Synthetic peptide
QIWPGDGDTNYNGKFKG

SEQ ID NO: 161 - protein, 15 aa, Artificial Sequence
  Description of Artificial Sequence: Synthetic peptide
RETTTVGRYYYAMDY